European Patent Application EP 4 786 583 A1, published August 5, 2026. Title: Method for specific degradation of G12V mutant protein of KRAS and composition thereof. Applicant: KANGWON NATIONAL UNIVERSITY RESEARCH & UNIVERSITY-INDUSTRY COOPERATION FOUNDATION. Application WO. The sequence listing filed with the application follows.

SEQUENCE LISTING (7 sequences)

SEQ ID NO: 1 - protein, 511 aa, synthetic construct
  REGION 1..511: note = iDAb-panRAS-NEDDHECT
MAEVQLLESGGGLVQPGGSLRLSCAASGFTFSTFSMNWVRQAPGKGLEWVSYISRTSKTIYYADSVKGRFTISRDNSKNTLYLQMNSLRAEDTAVYYCARGRFFDYWGQGTLVTVSSVDGGGGSLEVPYSREFKQKYDYFRKKLKKPADIPNRFEMKLHRNNIFEESYRRIMSVKRPDVLKARLWIEFESEKGLDYGGVAREWFFLLSKEMFNPYYGLFEYSATDNYTLQINPNSGLCNEDHLSYFTFIGRVAGLAVFHGKLLDGFFIRPFYKMMLGKQITLNDMESVDSEYYNSLKWILENDPTELDLMFCIDEENFGQTYQVDLKPNGSEIMVTNENKREYIDLVIQWRFVNRVQKQMNAFLEGFTELLPIDLIKIFDENELELLMCGLGDVDVNDWRQHSIYKNGYCPNHPVIQWFWKAVLLMDAEKRIRLLQFVTGTSRVPMNGFAELYGSNGPQLFTIEQWGSPEKLPRAHTCFNRLDLPPYETFEDLREKLLMAVENAQGFEGVD

SEQ ID NO: 2 - protein, 492 aa, synthetic construct
  REGION 1..492: note = 12VC1-NEDDHECT
MGSVSSVPTKLEVVAATPTSLLISWDAPAVTVFFYVITYGETGHGVGAFQAFKVPGSKSTATISGLKPGVDYTITVYARGYSKQGPYKPSPISINYRTVDGGGGSLEVPYSREFKQKYDYFRKKLKKPADIPNRFEMKLHRNNIFEESYRRIMSVKRPDVLKARLWIEFESEKGLDYGGVAREWFFLLSKEMFNPYYGLFEYSATDNYTLQINPNSGLCNEDHLSYFTFIGRVAGLAVFHGKLLDGFFIRPFYKMMLGKQITLNDMESVDSEYYNSLKWILENDPTELDLMFCIDEENFGQTYQVDLKPNGSEIMVTNENKREYIDLVIQWRFVNRVQKQMNAFLEGFTELLPIDLIKIFDENELELLMCGLGDVDVNDWRQHSIYKNGYCPNHPVIQWFWKAVLLMDAEKRIRLLQFVTGTSRVPMNGFAELYGSNGPQLFTIEQWGSPEKLPRAHTCFNRLDLPPYETFEDLREKLLMAVENAQGFEGVD

SEQ ID NO: 3 - protein, 543 aa, synthetic construct
  REGION 1..543: note = K55-NEDDHECT
DLGKKLLEAARAGQDDEVRILMANGADVNANDSAGHTPLHLAAKRGHLEIVEVLLKHGADVNAMDNTGFTPLHLAALRGHLEIVEVLLKNGADVNAQDRTGRTPLHLAAKLGHLEIVEVLLKNGADVNAQDKFGKTAFDISIDNGNEDLAEILQKLLEVPYSREFKQKYDYFRKKLKKPADIPNRFEMKLHRNNIFEESYRRIMSVKRPDVLKARLWIEFESEKGLDYGGVAREWFFLLSKEMFNPYYGLFEYSATDNYTLQINPNSGLCNEDHLSYFTFIGRVAGLAVFHGKLLDGFFIRPFYKMMLGKQITLNDMESVDSEYYNSLKWILENDPTELDLMFCIDEENFGQTYQVDLKPNGSEIMVTNENKREYIDLVIQWRFVNRVQKQMNAFLEGFTELLPIDLIKIFDENELELLMCGLGDVDVNDWRQHSIYKNGYCPNHPVIQWFWKAVLLMDAEKRIRLLQFVTGTSRVPMNGFAELYGSNGPQLFTIEQWGSPEKLPRAHTCFNRLDLPPYETFEDLREKLLMAVENAQGFEGVD

SEQ ID NO: 4 - protein, 551 aa, synthetic construct
  REGION 1..551: note = DP_KRAS-NEDDHECT
MDLGKKLLEAARAGQDDEVRILMANGADVNASDRWGWTPLHLAAWWGHLEIVEVLLKRGADVSAADLHGQSPLHLAAMVGHLEIVEVLLKYGADVNAKDTMGATPLHLAARSGHLEIVEELLKNGADMNAQDKFGKTTFDISTDNGNEDLAEILQKLVDGGGGSLEVPYSREFKQKYDYFRKKLKKPADIPNRFEMKLHRNNIFEESYRRIMSVKRPDVLKARLWIEFESEKGLDYGGVAREWFFLLSKEMFNPYYGLFEYSATDNYTLQINPNSGLCNEDHLSYFTFIGRVAGLAVFHGKLLDGFFIRPFYKMMLGKQITLNDMESVDSEYYNSLKWILENDPTELDLMFCIDEENFGQTYQVDLKPNGSEIMVTNENKREYIDLVIQWRFVNRVQKQMNAFLEGFTELLPIDLIKIFDENELELLMCGLGDVDVNDWRQHSIYKNGYCPNHPVIQWFWKAVLLMDAEKRIRLLQFVTGTSRVPMNGFAELYGSNGPQLFTIEQWGSPEKLPRAHTCFNRLDLPPYETFEDLREKLLMAVENAQGFEGVD

SEQ ID NO: 5 - protein, 543 aa, synthetic construct
  REGION 1..543: note = K27-NEDDHECT
DLGKKLLEAARAGQDDEVRILMANGADVNAHDTFGFTPLHLAALYGHLEIVEVLLKNGADVNADDSYGRTPLHLAAMRGHLEIVEVLLKYGADVNAADEEGRTPLHLAAKRGHLEIVEVLLKNGADVNAQDKFGKTAFDISIDNGNEDLAEILQKLLEVPYSREFKQKYDYFRKKLKKPADIPNRFEMKLHRNNIFEESYRRIMSVKRPDVLKARLWIEFESEKGLDYGGVAREWFFLLSKEMFNPYYGLFEYSATDNYTLQINPNSGLCNEDHLSYFTFIGRVAGLAVFHGKLLDGFFIRPFYKMMLGKQITLNDMESVDSEYYNSLKWILENDPTELDLMFCIDEENFGQTYQVDLKPNGSEIMVTNENKREYIDLVIQWRFVNRVQKQMNAFLEGFTELLPIDLIKIFDENELELLMCGLGDVDVNDWRQHSIYKNGYCPNHPVIQWFWKAVLLMDAEKRIRLLQFVTGTSRVPMNGFAELYGSNGPQLFTIEQWGSPEKLPRAHTCFNRLDLPPYETFEDLREKLLMAVENAQGFEGVD

SEQ ID NO: 6 - protein, 484 aa, synthetic construct
  REGION 1..484: note = NS1-NEDDHECT
GSVSSVPTKLEVVAATPTSLLISWDAPAVTVDYYVITYGETGGNSPVQKFEVPGSKSTATISGLKPGVDYTITVYAWGWHGQVYYYMGSPISINYRTLEVPYSREFKQKYDYFRKKLKKPADIPNRFEMKLHRNNIFEESYRRIMSVKRPDVLKARLWIEFESEKGLDYGGVAREWFFLLSKEMFNPYYGLFEYSATDNYTLQINPNSGLCNEDHLSYFTFIGRVAGLAVFHGKLLDGFFIRPFYKMMLGKQITLNDMESVDSEYYNSLKWILENDPTELDLMFCIDEENFGQTYQVDLKPNGSEIMVTNENKREYIDLVIQWRFVNRVQKQMNAFLEGFTELLPIDLIKIFDENELELLMCGLGDVDVNDWRQHSIYKNGYCPNHPVIQWFWKAVLLMDAEKRIRLLQFVTGTSRVPMNGFAELYGSNGPQLFTIEQWGSPEKLPRAHTCFNRLDLPPYETFEDLREKLLMAVENAQGFEGVD

SEQ ID NO: 7 - protein, 588 aa, synthetic construct
  REGION 1..588: note = RAF1_RBD_CRD-NEDDHECT
MEHIQGAWKTISNGFGFKDAVFDGSSCISPTIVQQFGYQRRASDDGKLTDPSKTSNTIRVFLPNKQRTVVNVRNGMSLHDCLMKALKVRGLQPECCAVFRLLHEHKGKKARLDWNTDAASLIGEELQVDFLDHVPLTTHNFARKTFLKLAFCDICQKFLLNGFRCQTCGYKFHEHCSTKVPTMCVDWSRRLNFGVDGGGGSLEVPYSREFKQKYDYFRKKLKKPADIPNRFEMKLHRNNIFEESYRRIMSVKRPDVLKARLWIEFESEKGLDYGGVAREWFFLLSKEMFNPYYGLFEYSATDNYTLQINPNSGLCNEDHLSYFTFIGRVAGLAVFHGKLLDGFFIRPFYKMMLGKQITLNDMESVDSEYYNSLKWILENDPTELDLMFCIDEENFGQTYQVDLKPNGSEIMVTNENKREYIDLVIQWRFVNRVQKQMNAFLEGFTELLPIDLIKIFDENELELLMCGLGDVDVNDWRQHSIYKNGYCPNHPVIQWFWKAVLLMDAEKRIRLLQFVTGTSRVPMNGFAELYGSNGPQLFTIEQWGSPEKLPRAHTCFNRLDLPPYETFEDLREKLLMAVENAQGFEGVD